European Patent Specification EP 3 974 027 B1, published October 23, 2024. Title: Stabilized Peptide of PACAP. Applicant: Senju Pharmaceutical Co., Ltd. The sequence listing filed with the application follows.

SEQUENCE LISTING (55 sequences)

SEQ ID NO: 1 - protein, 38 aa, Homo sapiens
HSDGIFTDSYSRYRKQMAVKKYLAAVLGKRYKQRVKNK

SEQ ID NO: 2 - protein, 27 aa, Homo sapiens
HSDGIFTDSYSRYRKQMAVKKYLAAVL

SEQ ID NO: 3 - protein, 27 aa, Artificial Sequence
  modified PACAP peptide
  MUTAGEN (2)..(2): Xaa is neutral amino acid
  MUTAGEN (5)..(5): Xaa is neutral amino acid
  MUTAGEN (7)..(7): Xaa is neutral amino acid
  MUTAGEN (9)..(9): Xaa is Ala, Ser, Aib, or b-cyano alanine
  MUTAGEN (11)..(11): Xaa is Ala, Ser, Aib, or b-cyano alanine
  MUTAGEN (16)..(16): Xaa is Gln or Ala
  MUTAGEN (17)..(17): Xaa is non-polar amino acid
HXDGXFXDXYXRYRKXXAVKKYLAAVL

SEQ ID NO: 4 - protein, 27 aa, Artificial Sequence
  modified PACAP peptide
  MUTAGEN (3)..(3): Xaa is amino acid wherein carboxy group of asparatic acid is substituted with tetrazole
  MUTAGEN (8)..(8): Xaa is amino acid wherein carboxy group of asparatic acid is substituted with tetrazole
  MOD_RES (27)..(27): AMIDATION
HSXGIFAXAYSRYRKQMAVKKYLAAVL

SEQ ID NO: 5 - protein, 27 aa, Artificial Sequence
  modified PACAP peptide
  MUTAGEN (3)..(3): Xaa is amino acid wherein carboxy group of asparatic acid is substituted with tetrazole
  MUTAGEN (8)..(8): Xaa is amino acid wherein carboxy group of asparatic acid is substituted with tetrazole
  MOD_RES (27)..(27): AMIDATION
HSXGIFAXSYARYRKQMAVKKYLAAVL

SEQ ID NO: 6 - protein, 27 aa, Artificial Sequence
  modified PACAP peptide
  MUTAGEN (3)..(3): Xaa is amino acid wherein carboxy group of asparatic acid is substituted with tetrazole
  MUTAGEN (8)..(8): Xaa is amino acid wherein carboxy group of asparatic acid is substituted with tetrazole
  MOD_RES (27)..(27): AMIDATION
HSXGIFAXAYARYRKQMAVKKYLAAVL

SEQ ID NO: 7 - protein, 27 aa, Artificial Sequence
  modified PACAP peptide
  MUTAGEN (3)..(3): Xaa is amino acid wherein carboxy group of asparatic acid is substituted with tetrazole
  MUTAGEN (8)..(8): Xaa is amino acid wherein carboxy group of asparatic acid is substituted with tetrazole
  MUTAGEN (9)..(9): Xaa is Aib
  MOD_RES (27)..(27): AMIDATION
HSXGIFAXXYSRYRKQMAVKKYLAAVL

SEQ ID NO: 8 - protein, 27 aa, Artificial Sequence
  modified PACAP peptide
  MUTAGEN (3)..(3): Xaa is amino acid wherein carboxy group of asparatic acid is substituted with tetrazole
  MUTAGEN (8)..(8): Xaa is amino acid wherein carboxy group of asparatic acid is substituted with tetrazole
  MUTAGEN (11)..(11): Xaa is Aib
  MOD_RES (27)..(27): AMIDATION
HSXGIFAXSYXRYRKQMAVKKYLAAVL

SEQ ID NO: 9 - protein, 27 aa, Artificial Sequence
  modified PACAP peptide
  MUTAGEN (3)..(3): Xaa is amino acid wherein carboxy group of asparatic acid is substituted with tetrazole
  MUTAGEN (8)..(8): Xaa is amino acid wherein carboxy group of asparatic acid is substituted with tetrazole
  MUTAGEN (9)..(9): Xaa is Aib
  MUTAGEN (11)..(11): Xaa is Aib
  MOD_RES (27)..(27): AMIDATION
HSXGIFAXXYXRYRKQMAVKKYLAAVL

SEQ ID NO: 10 - protein, 27 aa, Artificial Sequence
  modified PACAP peptide
  MUTAGEN (3)..(3): Xaa is amino acid wherein carboxy group of asparatic acid is substituted with tetrazole
  MUTAGEN (8)..(8): Xaa is amino acid wherein carboxy group of asparatic acid is substituted with tetrazole
  MUTAGEN (9)..(9): Xaa is Aib
  MUTAGEN (11)..(11): Xaa is Aib
  MOD_RES (27)..(27): AMIDATION
HSXGIFTXXYXRYRKQMAVKKYLAAVL

SEQ ID NO: 11 - protein, 24 aa, Artificial Sequence
  modified PACAP peptide
  MUTAGEN (3)..(3): Xaa is amino acid wherein carboxy group of asparatic acid is substituted with tetrazole
  MUTAGEN (8)..(8): Xaa is amino acid wherein carboxy group of asparatic acid is substituted with tetrazole
  MOD_RES (24)..(24): AMIDATION
HSXGIFTXSYSRYRKQMAVKKYLA

SEQ ID NO: 12 - protein, 26 aa, Artificial Sequence
  modified PACAP peptide
  MUTAGEN (3)..(3): Xaa is amino acid wherein carboxy group of asparatic acid is substituted with tetrazole
  MUTAGEN (8)..(8): Xaa is amino acid wherein carboxy group of asparatic acid is substituted with tetrazole
  MOD_RES (26)..(26): AMIDATION
HSXGIFTXSYSRYRKQMAVKKYLAAV

SEQ ID NO: 13 - protein, 27 aa, Artificial Sequence
  modified PACAP peptide
  MUTAGEN (3)..(3): Xaa is amino acid wherein carboxy group of asparatic acid is substituted with sulfoxy
  MUTAGEN (8)..(8): Xaa is amino acid wherein carboxy group of asparatic acid is substituted with sulfoxy
  MOD_RES (27)..(27): AMIDATION
HSXGIFTXSYSRYRKQLAVKKYLAAVL

SEQ ID NO: 14 - protein, 27 aa, Artificial Sequence
  modified PACAP peptide
  MUTAGEN (3)..(3): Xaa is amino acid wherein carboxy group of asparatic acid is substituted with sulfoxy
  MUTAGEN (8)..(8): Xaa is amino acid wherein carboxy group of asparatic acid is substituted with sulfoxy
  MUTAGEN (17)..(17): Xaa is Nle
  MOD_RES (27)..(27): AMIDATION
HSXGIFTXSYSRYRKQXAVKKYLAAVL

SEQ ID NO: 15 - protein, 28 aa, Artificial Sequence
  modified PACAP peptide
  MUTAGEN (4)..(4): Xaa is amino acid wherein carboxy group of asparatic acid is substituted with tetrazole
  MUTAGEN (9)..(9): Xaa is amino acid wherein carboxy group of asparatic acid is substituted with tetrazole
  MOD_RES (28)..(28): AMIDATION
MHSXGIFTXSYSRYRKQLAVKKYLAAVL

SEQ ID NO: 16 - protein, 27 aa, Artificial Sequence
  modified PACAP peptide
  MUTAGEN (3)..(3): Xaa is D-amino acid wherein carboxy group of asparatic acid is substituted with tetrazole
  MUTAGEN (8)..(8): Xaa is D-amino acid wherein carboxy group of asparatic acid is substituted with tetrazole
  MUTAGEN (17)..(17): Xaa is Nle
  MOD_RES (27)..(27): AMIDATION
HSXGIFTXSYSRYRKQXAVKKYLAAVL

SEQ ID NO: 17 - protein, 27 aa, Artificial Sequence
  modified PACAP peptide
  MUTAGEN (3)..(3): Xaa is amino acid wherein carboxy group of asparatic acid is substituted with tetrazole
  MUTAGEN (8)..(8): Xaa is D- amino acid wherein carboxy group of asparatic acid is substituted with tetrazole
  MUTAGEN (17)..(17): Xaa is Nle
  MOD_RES (27)..(27): AMIDATION
HSXGIFTXSYSRYRKQXAVKKYLAAVL

SEQ ID NO: 18 - protein, 27 aa, Artificial Sequence
  modified PACAP peptide
  MUTAGEN (3)..(3): Xaa is D-amino acid wherein carboxy group of asparatic acid is substituted with tetrazole
  MUTAGEN (8)..(8): Xaa is amino acid wherein carboxy group of asparatic acid is substituted with tetrazole
  MUTAGEN (17)..(17): Xaa is Nle
  MOD_RES (27)..(27): AMIDATION
HSXGIFTXSYSRYRKQXAVKKYLAAVL

SEQ ID NO: 19 - protein, 27 aa, Artificial Sequence
  modified PACAP peptide
  MUTAGEN (3)..(3): Xaa is amino acid wherein carboxy group of asparatic acid is substituted with tetrazole
  MUTAGEN (8)..(8): Xaa is amino acid wherein carboxy group of glutamic acid is substituted with tetrazole
  MUTAGEN (17)..(17): Xaa is Nle
  MOD_RES (27)..(27): AMIDATION
HSXGIFTXSYSRYRKQXAVKKYLAAVL

SEQ ID NO: 20 - protein, 27 aa, Artificial Sequence
  modified PACAP peptide
  MOD_RES (1)..(1): PROPYONYLATION
  MUTAGEN (3)..(3): Xaa is amino acid wherein carboxy group of asparatic acid is substituted with tetrazole
  MUTAGEN (8)..(8): Xaa is amino acid wherein carboxy group of asparatic acid is substituted with tetrazole
  MUTAGEN (17)..(17): Xaa is Nle
  MOD_RES (27)..(27): AMIDATION
HSXGIFTXSYSRYRKQXAVKKYLAAVL

SEQ ID NO: 21 - protein, 27 aa, Artificial Sequence
  modified PACAP peptide
  MOD_RES (1)..(1): BUTYRYLATION
  MUTAGEN (3)..(3): Xaa is amino acid wherein carboxy group of asparatic acid is substituted with tetrazole
  MUTAGEN (8)..(8): Xaa is amino acid wherein carboxy group of asparatic acid is substituted with tetrazole
  MUTAGEN (17)..(17): Xaa is Nle
  MOD_RES (27)..(27): AMIDATION
HSXGIFTXSYSRYRKQXAVKKYLAAVL

SEQ ID NO: 22 - protein, 27 aa, Artificial Sequence
  modified PACAP peptide
  MOD_RES (1)..(1): ISOBUTYRYLATION
  MUTAGEN (3)..(3): Xaa is amino acid wherein carboxy group of asparatic acid is substituted with tetrazole
  MUTAGEN (8)..(8): Xaa is amino acid wherein carboxy group of asparatic acid is substituted with tetrazole
  MUTAGEN (17)..(17): Xaa is Nle
  MOD_RES (27)..(27): AMIDATION
HSXGIFTXSYSRYRKQXAVKKYLAAVL

SEQ ID NO: 23 - protein, 27 aa, Artificial Sequence
  modified PACAP peptide
  MOD_RES (1)..(1): PENTANOYLATION
  MUTAGEN (3)..(3): Xaa is amino acid wherein carboxy group of asparatic acid is substituted with tetrazole
  MUTAGEN (8)..(8): Xaa is amino acid wherein carboxy group of asparatic acid is substituted with tetrazole
  MUTAGEN (17)..(17): Xaa is Nle
  MOD_RES (27)..(27): AMIDATION
HSXGIFTXSYSRYRKQXAVKKYLAAVL

SEQ ID NO: 24 - protein, 27 aa, Artificial Sequence
  modified PACAP peptide
  MOD_RES (1)..(1): ISOPENTANOYLATION
  MUTAGEN (3)..(3): Xaa is amino acid wherein carboxy group of asparatic acid is substituted with tetrazole
  MUTAGEN (8)..(8): Xaa is amino acid wherein carboxy group of asparatic acid is substituted with tetrazole
  MUTAGEN (17)..(17): Xaa is Nle
  MOD_RES (27)..(27): AMIDATION
HSXGIFTXSYSRYRKQXAVKKYLAAVL

SEQ ID NO: 25 - protein, 27 aa, Artificial Sequence
  modified PACAP peptide
  MOD_RES (1)..(1): ACETYLATION
  MUTAGEN (3)..(3): Xaa is amino acid wherein carboxy group of asparatic acid is substituted with oxadiazolone
  MUTAGEN (8)..(8): Xaa is amino acid wherein carboxy group of asparatic acid is substituted with oxadiazolone
  MUTAGEN (17)..(17): Xaa is Nle
  MOD_RES (27)..(27): AMIDATION
HSXGIFTXSYSRYRKQXAVKKYLAAVL

SEQ ID NO: 26 - protein, 27 aa, Artificial Sequence
  modified PACAP peptide
  MOD_RES (1)..(1): ACETYLATION
  MUTAGEN (3)..(3): Xaa is amino acid wherein carboxy group of asparatic acid is substituted with tetrazole
  MUTAGEN (8)..(8): Xaa is amino acid wherein carboxy group of asparatic acid is substituted with tetrazole
  MOD_RES (27)..(27): AMIDATION
HSXGAFTXSYSRYRKQLAVKKYLAAVL

SEQ ID NO: 27 - protein, 27 aa, Artificial Sequence
  modified PACAP peptide
  MOD_RES (1)..(1): ACETYLATION
  MUTAGEN (3)..(3): Xaa is amino acid wherein carboxy group of asparatic acid is substituted with tetrazole
  MUTAGEN (8)..(8): Xaa is amino acid wherein carboxy group of asparatic acid is substituted with tetrazole
  MOD_RES (27)..(27): AMIDATION
HSXGIFAXSYSRYRKQLAVKKYLAAVL

SEQ ID NO: 28 - protein, 27 aa, Artificial Sequence
  modified PACAP peptide
  MOD_RES (1)..(1): ACETYLATION
  MUTAGEN (3)..(3): Xaa is amino acid wherein carboxy group of asparatic acid is substituted with tetrazole
  MUTAGEN (8)..(8): Xaa is amino acid wherein carboxy group of asparatic acid is substituted with tetrazole
  MOD_RES (27)..(27): AMIDATION
HAXGIFAXSYSRYRKQLAVKKYLAAVL

SEQ ID NO: 29 - protein, 27 aa, Artificial Sequence
  modified PACAP peptide
  MOD_RES (1)..(1): ACETYLATION
  MUTAGEN (3)..(3): Xaa is amino acid wherein carboxy group of asparatic acid is substituted with tetrazole
  MUTAGEN (8)..(8): Xaa is amino acid wherein carboxy group of asparatic acid is substituted with tetrazole
  MOD_RES (27)..(27): AMIDATION
HAXGIFTXSYSRYRKALAVKKYLAAVL

SEQ ID NO: 30 - protein, 27 aa, Artificial Sequence
  modified PACAP peptide
  MOD_RES (1)..(1): ACETYLATION
  MUTAGEN (3)..(3): Xaa is amino acid wherein carboxy group of asparatic acid is substituted with tetrazole
  MUTAGEN (8)..(8): Xaa is amino acid wherein carboxy group of asparatic acid is substituted with tetrazole
  MOD_RES (27)..(27): AMIDATION
HSXGIFAXAYSRYRKQLAVKKYLAAVL

SEQ ID NO: 31 - protein, 27 aa, Artificial Sequence
  modified PACAP peptide
  MOD_RES (1)..(1): ACETYLATION
  MUTAGEN (3)..(3): Xaa is amino acid wherein carboxy group of asparatic acid is substituted with tetrazole
  MUTAGEN (8)..(8): Xaa is amino acid wherein carboxy group of asparatic acid is substituted with tetrazole
  MOD_RES (27)..(27): AMIDATION
HSXGIFAXSYSRYRKALAVKKYLAAVL

SEQ ID NO: 32 - protein, 27 aa, Artificial Sequence
  modified PACAP peptide
  MOD_RES (1)..(1): ACETYLATION
  MUTAGEN (3)..(3): Xaa is amino acid wherein carboxy group of asparatic acid is substituted with tetrazole
  MUTAGEN (8)..(8): Xaa is amino acid wherein carboxy group of asparatic acid is substituted with tetrazole
  MOD_RES (27)..(27): AMIDATION
HSXGIFAXSYSRYRKQAAVKKYLAAVL

SEQ ID NO: 33 - protein, 27 aa, Artificial Sequence
  modified PACAP peptide
  MOD_RES (1)..(1): ACETYLATION
  MUTAGEN (3)..(3): Xaa is amino acid wherein carboxy group of asparatic acid is substituted with tetrazole
  MUTAGEN (8)..(8): Xaa is amino acid wherein carboxy group of asparatic acid is substituted with tetrazole
  MOD_RES (27)..(27): AMIDATION
HAXGIFAXAYSRYRKAAAVKKYLAAVL

SEQ ID NO: 34 - protein, 27 aa, Artificial Sequence
  modified PACAP peptide
  MUTAGEN (3)..(3): Xaa is amino acid wherein carboxy group of asparatic acid is substituted with tetrazole
  MUTAGEN (8)..(8): Xaa is amino acid wherein carboxy group of asparatic acid is substituted with tetrazole
  MUTAGEN (11)..(11): Xaa is b-cyano alanine
  MOD_RES (27)..(27): AMIDATION
HSXGIFAXSYXRYRKQMAVKKYLAAVL

SEQ ID NO: 35 - protein, 27 aa, Artificial Sequence
  modified PACAP peptide
  MUTAGEN (3)..(3): Xaa is amino acid wherein carboxy group of asparatic acid is substituted with tetrazole
  MUTAGEN (8)..(8): Xaa is amino acid wherein carboxy group of asparatic acid is substituted with tetrazole
  MUTAGEN (9)..(9): Xaa is b-cyano alanine
  MUTAGEN (11)..(11): Xaa is b-cyano alanine
  MOD_RES (27)..(27): AMIDATION
HSXGIFTXXYXRYRKQMAVKKYLAAVL

SEQ ID NO: 36 - protein, 27 aa, Artificial Sequence
  modified PACAP peptide
  MUTAGEN (3)..(3): Xaa is amino acid wherein carboxy group of glutamic acid is substituted with tetrazole
  MUTAGEN (8)..(8): Xaa is amino acid wherein carboxy group of asparatic acid is substituted with tetrazole
  MUTAGEN (17)..(17): Xaa is Nle
  MOD_RES (27)..(27): AMIDATION
HSXGIFTXSYSRYRKQXAVKKYLAAVL

SEQ ID NO: 37 - protein, 27 aa, Artificial Sequence
  modified PACAP peptide
  MUTAGEN (3)..(3): Xaa is amino acid wherein carboxy group of glutamic acid is substituted with tetrazole
  MUTAGEN (8)..(8): Xaa is amino acid wherein carboxy group of glutamic acid is substituted with tetrazole
  MUTAGEN (17)..(17): Xaa is Nle
  MOD_RES (27)..(27): AMIDATION
HSXGIFTXSYSRYRKQXAVKKYLAAVL

SEQ ID NO: 38 - protein, 27 aa, Artificial Sequence
  modified PACAP peptide
  MUTAGEN (3)..(3): Xaa is amino acid wherein carboxy group of homoglutamic acid is substituted with tetrazole
  MUTAGEN (8)..(8): Xaa is amino acid wherein carboxy group of asparatic acid is substituted with tetrazole
  MUTAGEN (17)..(17): Xaa is Nle
  MOD_RES (27)..(27): AMIDATION
HSXGIFTXSYSRYRKQXAVKKYLAAVL

SEQ ID NO: 39 - protein, 27 aa, Artificial Sequence
  modified PACAP peptide
  MUTAGEN (3)..(3): Xaa is amino acid wherein carboxy group of asparatic acid is substituted with tetrazole
  MUTAGEN (8)..(8): Xaa is amino acid wherein carboxy group of homoglutamic acid is substituted with tetrazole
  MUTAGEN (17)..(17): Xaa is Nle
  MOD_RES (27)..(27): AMIDATION
HSXGIFTXSYSRYRKQXAVKKYLAAVL

SEQ ID NO: 40 - protein, 27 aa, Artificial Sequence
  modified PACAP peptide
  MUTAGEN (3)..(3): Xaa is amino acid wherein carboxy group of homoglutamic acid is substituted with tetrazole
  MUTAGEN (8)..(8): Xaa is amino acid wherein carboxy group of homoglutamic acid is substituted with tetrazole
  MUTAGEN (17)..(17): Xaa is Nle
  MOD_RES (27)..(27): AMIDATION
HSXGIFTXSYSRYRKQXAVKKYLAAVL

SEQ ID NO: 41 - protein, 27 aa, Artificial Sequence
  modified PACAP peptide
  MUTAGEN (3)..(3): Xaa is amino acid wherein carboxy group of glutamic acid is substituted with tetrazole
  MUTAGEN (8)..(8): Xaa is amino acid wherein carboxy group of homoglutamic acid is substituted with tetrazole
  MUTAGEN (17)..(17): Xaa is Nle
  MOD_RES (27)..(27): AMIDATION
HSXGIFTXSYSRYRKQXAVKKYLAAVL

SEQ ID NO: 42 - protein, 27 aa, Artificial Sequence
  modified PACAP peptide
  MUTAGEN (3)..(3): Xaa is amino acid wherein carboxy group of homoglutamic acid is substituted with tetrazole
  MUTAGEN (8)..(8): Xaa is amino acid wherein carboxy group of glutamic acid is substituted with tetrazole
  MUTAGEN (17)..(17): Xaa is Nle
  MOD_RES (27)..(27): AMIDATION
HSXGIFTXSYSRYRKQXAVKKYLAAVL

SEQ ID NO: 43 - protein, 11 aa, Homo sapiens
GKRYKQRVKNK

SEQ ID NO: 44 - protein, 10 aa, Homo sapiens
GKRYKQRVKN

SEQ ID NO: 45 - protein, 9 aa, Homo sapiens
GKRYKQRVK

SEQ ID NO: 46 - protein, 8 aa, Homo sapiens
GKRYKQRV

SEQ ID NO: 47 - protein, 7 aa, Homo sapiens
GKRYKQR

SEQ ID NO: 48 - protein, 6 aa, Homo sapiens
GKRYKQ

SEQ ID NO: 49 - protein, 5 aa, Homo sapiens
GKRYK

SEQ ID NO: 50 - protein, 4 aa, Homo sapiens
GKRY

SEQ ID NO: 51 - protein, 27 aa, Artificial Sequence
  modified PACAP peptide
  MOD_RES (1)..(1): ACETYLATION
HSDGIFTDSYSRYRKQMAVKKYLAAVL

SEQ ID NO: 52 - protein, 27 aa, Artificial Sequence
  modified PACAP peptide
  MUTAGEN (3)..(3): Xaa is amino acid wherein carboxy group of asparatic acid is substituted with tetrazole
  MUTAGEN (8)..(8): Xaa is amino acid wherein carboxy group of asparatic acid is substituted with tetrazole
  MUTAGEN (17)..(17): Xaa is Nle
HSXGIFTXSYSRYRKQXAVKKYLAAVL

SEQ ID NO: 53 - protein, 27 aa, Artificial Sequence
  modified PACAP peptide
  MUTAGEN (3)..(3): Xaa is amino acid wherein carboxy group of asparatic acid is substituted with tetrazole
  MUTAGEN (8)..(8): Xaa is amino acid wherein carboxy group of asparatic acid is substituted with tetrazole
HSXGIFTXSYSRYRKQLAVKKYLAAVL

SEQ ID NO: 54 - protein, 27 aa, Artificial Sequence
  modified PACAP peptide
  MOD_RES (1)..(1): ACETYLATION
  MUTAGEN (3)..(3): Xaa is amino acid wherein carboxy group of asparatic acid is substituted with tetrazole
  MUTAGEN (8)..(8): Xaa is amino acid wherein carboxy group of asparatic acid is substituted with tetrazole
  MUTAGEN (17)..(17): Xaa is Nle
HSXGIFTXSYSRYRKQXAVKKYLAAVL

SEQ ID NO: 55 - protein, 27 aa, Artificial Sequence
  modified PACAP peptide
  MOD_RES (1)..(1): ACETYLATION
  MUTAGEN (3)..(3): Xaa is amino acid wherein carboxy group of asparatic acid is substituted with tetrazole
  MUTAGEN (8)..(8): Xaa is amino acid wherein carboxy group of asparatic acid is substituted with tetrazole
HSXGIFTXSYSRYRKQLAVKKYLAAVL